European Patent Application EP 4 772 530 A1, published July 8, 2026. Title: 一种靶向生长抑素受体的肽、偶联药物及其应用. Applicant: 主流源生物科技(上海)有限公司. The sequence listing filed with the application follows.

SEQUENCE LISTING (6 sequences)

SEQ ID NO: 1 - protein, 13 aa, synthetic construct
RXFCXWKTCTXRX

SEQ ID NO: 2 - protein, 14 aa, synthetic construct
XRXFCXWKTCTXRX

SEQ ID NO: 3 - protein, 14 aa, synthetic construct
RRLFCYWKTCTWRD

SEQ ID NO: 4 - protein, 14 aa, synthetic construct
RRLFCFWYTCTWRD

SEQ ID NO: 5 - protein, 13 aa, synthetic construct
GRRFCYWKTCTDR

SEQ ID NO: 6 - protein, 14 aa, synthetic construct
RRLFCYWKTCTWRD